European Patent Specification EP 3 962 559 B1, published April 16, 2025. Title: METHODS AND COMPOSITIONS FOR TREATING CHRONIC INFLAMMATORY INJURY, METAPLASIA, DYSPLASIA AND CANCERS OF EPITHELIAL TISSUES. Applicant: UNIVERSITY OF HOUSTON SYSTEM THE BOARD OF REGENTS OF THE UNIVERSITY OF TEXAS SYSTEM TRACT PHARMACEUTICALS, INC. The sequence listing filed with the application follows.

SEQUENCE LISTING (2 sequences)

SEQ ID NO: 1 - DNA, 63 bp, Artificial sequence
  Synthetic nucleic acid
cagggaagtttcgagaagtcctatagtgaagccacagatgtataggactctcgaacttccctt

SEQ ID NO: 2 - DNA, 63 bp, Artificial sequence
  Synthetic nucleic acid
acaccagcagtagcaacagcaatagtgaagccacagatgtattgctgttgctactgctggtgg